European Patent Specification EP 3 443 127 B1, published October 11, 2023. Title: Freeze-resistant yeast and uses thereof. Applicant: NextFerm Technologies Ltd. The sequence listing filed with the application follows.

SEQUENCE LISTING (9 sequences)

SEQ ID NO: 1 - DNA, 20 bp, Artificial Sequence
  Primer
ctgtatggttcgccgtttat

SEQ ID NO: 2 - DNA, 22 bp, Artificial Sequence
  Primer
ggtaatctgtgggatgtaactg

SEQ ID NO: 3 - DNA, 18 bp, Artificial Sequence
  Primer
attgcctctcagtatcgt

SEQ ID NO: 4 - DNA, 19 bp, Artificial Sequence
  Primer
cacaaatcttccaaaccac

SEQ ID NO: 5 - DNA, 20 bp, Artificial Sequence
  Primer
cgctgtagcaaagcaaaaag

SEQ ID NO: 6 - DNA, 19 bp, Artificial Sequence
  Primer
gcaatgaccgtaggagtga

SEQ ID NO: 7 - DNA, 604 bp, Saccharomyces cerevisiae
ctgtatggttcgccgtttattttctaagcaccgttttttattcatatttttataatgcaactcctatagaatatagatgtttcgtgtttttaattcctgctatgactttgtgtcaatggtatgtgaactaacaactgtgtggtagtttgggatggtacgtaaaggtgttcgtgattatataagcaatcttaaaatatttgtatcgcaccatgaggtgcccaataatgaaatgaaaattactattatgaactatactaaaaagatgaaacttttttatcaatcccaggttcttttacttattatttttggatataagaacaaaatcggatttcccatgctttttctcaatgtctatatgaaatcttttcgaaacagccagtacatgtaacaattatgatacgaacttgatcggtaacccataaataacaggagctgcgccgttcaagtaacgtagatggcatacacctctagatttagagacggcatatgaaacagataggctattaccattcaaatcgtcagtattacagcgaaatcccatcttttcaaaaagttcctcgctaaatttatcaatatctttgtcagttacatcccacagattacc

SEQ ID NO: 8 - DNA, 372 bp, Saccharomyces cerevisiae
attgcctctcagtatcgtaattctatgtgggtatctgactttcatggcaactaggtaagatacagtttcaacagaataatatcctctatccacgtaatcacccatgaaaaggtaattggtgtcaggacaaggaccaccaatcttgaaaagttctaacaagtcatggaattgaccgtgtacgtcaccacaaatagtaacaggcacattaattggtttaacattttcctcgaactgcaacacgtccaccgccattttacatagtcgtgctacatcgtcttctgatagtggctcgcatttactcaaatgctcaatccattggtcaagctgatttatatttgtgttattcagttctagtggtttggaagatttgtg

SEQ ID NO: 9 - DNA, 616 bp, Saccharomyces cerevisiae
cgctgtagcaaagcaaaaagtttctgattcaaaataagtcacctactcttagcgcatttttattgtatataaaggcatttaatgtaatttatagagcattataaatcgtaacaactactgcagtatgagtttcatgaattcatttctcgatatcttatgaatatacacaggtatatatgtatattcatgttaaacgcctttcgaattgttcgttggctttttttgtgaaattatctcgggaaaagggcgaaattatatcgttttgccgttgatattttgaaaaggaataaaagatcatgaaaaaaataagaaaggcaattcgacgcatttctctcagcaagctattctttacttttgaagaataaaatatttgagtaaaaaggttaagacaatatagtcggaagcagttctgcgggatctgaaggaattgcggaataatgagatttcacgatagtatacttatcttcttttctttggcatcgctttatcaacatgttcatggtgcaagacaagtcgttcgtccaaaggagaaaatgactacttcagaagaagttaaaccttggttacgtacggtttatggaagtcaaaaagaattagtcactcctacggtcattgc